European Patent Specification EP 3 902 572 B1, published March 4, 2026. Title: A BONE REGENERATION MATERIAL HAVING A COTTON-WOOL LIKE STRUCTURE FORMED OF A PLURALITY OF ELECTROSPUN FIBERS. Applicant: ORTHOREBIRTH CO., LTD. THERADAPTIVE, INC. The sequence listing filed with the application follows.

SEQUENCE LISTING (22 sequences)

SEQ ID NO: 1 - protein, 12 aa, Artificial Sequence
  Synthetic
LLADTTHHRPWT

SEQ ID NO: 2 - protein, 12 aa, Artificial Sequence
  Synthetic
GQVLPTTTPSSP

SEQ ID NO: 3 - protein, 12 aa, Artificial Sequence
  Synthetic
VPQHPYPVPSHK

SEQ ID NO: 4 - protein, 12 aa, Artificial Sequence
  Synthetic
HNMAPATLHPLP

SEQ ID NO: 5 - protein, 12 aa, Artificial Sequence
  Synthetic
QSFASLTNPRVL

SEQ ID NO: 6 - protein, 12 aa, Artificial Sequence
  Synthetic
HTTPTTTYAAPP

SEQ ID NO: 7 - protein, 12 aa, Artificial Sequence
  Synthetic
QYGVVSHLTHTP

SEQ ID NO: 8 - protein, 12 aa, Artificial Sequence
  Synthetic
TMSNPITSLISV

SEQ ID NO: 9 - protein, 12 aa, Artificial Sequence
  Synthetic
IGRISTHAPLHP

SEQ ID NO: 10 - protein, 12 aa, Artificial Sequence
  Synthetic
MNDPSPWLRSPR

SEQ ID NO: 11 - protein, 12 aa, Artificial Sequence
  Synthetic
QSLGSMFQEGHR

SEQ ID NO: 12 - protein, 12 aa, Artificial Sequence
  Synthetic
KPLFTRYGDVAI

SEQ ID NO: 13 - protein, 12 aa, Artificial Sequence
  Synthetic
MPFGARILSLPN

SEQ ID NO: 14 - protein, 12 aa, Artificial Sequence
  Synthetic
QLQLSNSMSSLS

SEQ ID NO: 15 - protein, 12 aa, Artificial Sequence
  Synthetic
TMNMPAKIFAAM

SEQ ID NO: 16 - protein, 12 aa, Artificial Sequence
  Synthetic
EPTKEYTTSYHR

SEQ ID NO: 17 - protein, 12 aa, Artificial sequence
  Synthetic
DLNELYLRSLRA

SEQ ID NO: 18 - protein, 12 aa, Artificial Sequence
  Synthetic
DYDSTHGAVFRL

SEQ ID NO: 19 - protein, 12 aa, Artificial Sequence
  Synthetic
SKHERYPQSPEM

SEQ ID NO: 20 - protein, 12 aa, Artificial Sequence
  Synthetic
HTHSSDGSLLGN

SEQ ID NO: 21 - protein, 12 aa, Artificial Sequence
  Synthetic
NYDSMSEPRSHG

SEQ ID NO: 22 - protein, 12 aa, Artificial Sequence
  Synthetic
ANPIISVQTAMD